European Patent Application EP 4 778 937 A1, published July 22, 2026. Title: 特异性TIGIT肽段. Applicant: 重庆精准生物技术有限公司. The sequence listing filed with the application follows.

SEQUENCE LISTING (53 sequences)

SEQ ID NO: 1 - protein, 120 aa, synthetic construct
MMTGTIETTGNISAEKGGSIILQCHLSSTTAQVTQVNWEQQDQLLAICNADLGWHISPSFKDRVAPGPGLGLTLQSLTVNDTGEYFCIYHTYPDGTYTGRIFLEVLESSVAEHGARFQIP

SEQ ID NO: 2 - protein, 120 aa, synthetic construct
MMTGTIETTGNISAEKGGSIILQCHLSSTTAQVTQVDWEQQDQLLAISNADLGWHISPSFKDRVAPGPGLGLTLQSLTVNDTGEYFCIYHTYPDGTYTGRIFLEVLESSVAEHGARFQIP

SEQ ID NO: 3 - protein, 120 aa, synthetic construct
MMTGTIETTGNISAEKGGSIILQCHLSSTTAQVTQVDWEQQDQLLAIYNADLGWHISPSFKDRVAPGPGLGLTLQSLTVNDTGEYFCIYHTYPDGTYTGRIFLEVLESSVAEHGARFQIP

SEQ ID NO: 4 - protein, 120 aa, synthetic construct
MMTGTIETTGNISAEKGGSIILQCHLSSTTAQVTQVDWEQQDQLLAIYNADLGWHISPSFKDRVAPGPGLGLTLQPLTVNDTGEYFCIYHTYPDGTYTGRIFLEVLESSEAEHGARFQIP

SEQ ID NO: 5 - protein, 120 aa, synthetic construct
MMTGTIETTGNISAEKGGSIIFQCHLSSTTAQVTQVDWGQQDQLLAIYNADLGWHISPSFKDRVAPGPGLGLTLQSLTVNDTGEYFCIYHTYPDGTYTGRIFLEVLESSVAEHGARFQIP

SEQ ID NO: 6 - protein, 120 aa, synthetic construct
MMTGTIETTGNISAEKGGSIILQCHLSSTTAQVTQVDWEQQDQLLAIWNADLGWHISPSFKDRVAPGPGLGLTLQSLTVNDTGEYFCIYHTYPDGTYTGRIFLEVLESSVAEHGARFQIP

SEQ ID NO: 7 - protein, 120 aa, synthetic construct
MMTGTIETTGNISAEKGGSIILQCHLSSTTAQVTQVNWEQQDQLLAIWNADLGWHISPSFKDRVAPGPGLGLTLQSLTVNDTGEYFCIYHTYPDGTYTGRIFLEVLESSVAEHGARFQIP

SEQ ID NO: 8 - protein, 120 aa, synthetic construct
MMTGTIETTGNISAEKGGSIILQCHLSSTTAQVTQVDWEQQDQLLAICNADLGWHISPSFKDRVAPGPGLGLTLQSLTVNDTGEYFCIYHTYPDGTYTGRIFLEVLESSVAEHGARFQIP

SEQ ID NO: 9 - protein, 120 aa, synthetic construct
MMTGTIETTGNISAEKGGSTILQCHLSSTTAQVTQVDWKQQDQFLAIWNADLGWHISPSFKDRVAPGPGLGLTLQSLTVNDTGEYFCIYHTYPDGTYTGRIFLEVQESSVAEHGARFQIP

SEQ ID NO: 10 - protein, 120 aa, synthetic construct
MMTGTIETTGNLSAEKGGSIILQCHLSSTTAQVTQVEWEQQDQLLAIWNADLGWHISPSFKDRVAPGPGLDLTLQSLTVNDTGEYFCIYHTYPDGTYTGRISLEVLESSVAEHGARFQIP

SEQ ID NO: 11 - protein, 120 aa, synthetic construct
MMTGTIETTGNISAEKGGSTILQCHLSSTTAQVTQVDWEQQGQLLAIWNADLGWHISPSFKDRVAPGPGQGLTLQSLTVNDTGEYFCIYHTYPDGTYTGRIFLEVLESSVAEHGARFQIP

SEQ ID NO: 12 - protein, 120 aa, synthetic construct
MMTGTIETTGNISAEKGGSIFLQCHLSSTTAQVSQVEWKQQDQLLAIWNADLGWHISPSFKDRVAPGPGPGLTLQSLTVYDTGEYFCIYHTYPDGTYTGRTFLEVLESSAAEHGARFQIP

SEQ ID NO: 13 - protein, 120 aa, synthetic construct
MMTGTIETSGNISAEKGGSIILQCHLSSTTAQVTQVDWVQQDQLLAIWNADLGWHISPSFRDRVAPGPGLGLTLQSLTVNDTGEYFCIYHTYPDGTYTGRTFLEVLESSVAEHGARFQIP

SEQ ID NO: 14 - protein, 120 aa, synthetic construct
MMTGTIETTGNISAEKGGSTILQCHLSSTTAQVTQVDWKQQDQLLAIWNADLGWHISPSFKDRVAPGPGLGLTLQSLTVNDTGEYFCIYHTYPDGTYTGRIFLEVLESSVAEHGARFQIP

SEQ ID NO: 15 - protein, 120 aa, synthetic construct
MMTGTIETTGNISAEKGGSIILQCHLSSTTAQVTQVDWEQQDQLLAIYNADLGWHISPSFKDRVAPGPGLGLTLQSLTVNDTGEYSCIYHTYPDGTYTGRIFLEVLESSVAEYGARFQIP

SEQ ID NO: 16 - protein, 120 aa, synthetic construct
MWTGTIETTGNISAEKGGSIILQCHLSSTTAQVTQVDWEQQDQLLAIWNADLGWHFSPSFKDRVAPGPGLGLTLQSLTVNDTGEYFCIYHTYPDGTYTGRIFLEVLESSVAEHGARFQIP

SEQ ID NO: 17 - protein, 120 aa, synthetic construct
MMTGTIETTGNNSVEKGGSIFLQCHLSSTTAQVTQVDWKQQDQLLAIWNADLGWHISPSFKDRVAPGPGQGLTLQSLTVNDTGEYFCIYHTYPDGTYTGRIFLEVLESSVAEHGARFQIP

SEQ ID NO: 18 - protein, 120 aa, synthetic construct
MMTGTIETTGNISAEKGGSIILQCHLSSTTAQVTQVDWEQQDQLLAIWNADLGWHIPPSFKDRVAPGPGLGLTLQSLTVNDTGEYSCIYHTYPDGTYTGRIFLEVLESSVAEHGARFQIP

SEQ ID NO: 19 - protein, 120 aa, synthetic construct
MTTGTIETTGNISAEKGGSIILQCHLSSTTAQVTQVDWKQQDQLLAIWNADLGWHISPSFKDRVAPGPGLGLTLQSLTVNDTGEYLCIYHTYPDGTYTGRIFLEVLESSVAEHGARFQIP

SEQ ID NO: 20 - protein, 120 aa, synthetic construct
MMTGTIETTGNISAEKGGSTILQCHLSSTTAQVTQVDWEQQDQLLAIWNADLGWHISPSFKDRVAPGPGLGLTLQSLTVNDTGEYFCIYHTYPDGTYTGRIFLEVLESSVAEHGARFQIP

SEQ ID NO: 21 - protein, 120 aa, synthetic construct
MMTGTIETTGNISAEKGGSIILQCHLSSTTAQVTQVDWEQQDQLLAIWNADLGWHISPSFKDRVAPGPGLGLTLQSLTENDTGEYFCIYHTYPDGTYTGRIFLEVLESSVAEHGARFQIP

SEQ ID NO: 22 - protein, 120 aa, synthetic construct
MMTGTIETTGNISAEKGGSIILQCHLSSTTAQVTQVNWEQQDQLLAISNADLGWHISPSFKDRVAPGPGLGLTLQSLTVNDTGEYFCIYHTYPDGTYTGRIFLEVLESSVAEHGARFQIP

SEQ ID NO: 23 - protein, 120 aa, synthetic construct
MMTGTIETTGNISAEKGGSIILQCHLSSTTAQVTQVNWEQQDQLLAIRNADLGWHISPSFKDRVAPGPGLGLTLQSLTVNDTGEYFCIYHTYPDGTYTGRIFLEVLESSVAEHGARFQIP

SEQ ID NO: 24 - protein, 120 aa, synthetic construct
MMTGTIETTGNISAEKGGSIILQCHLSSTTAQVTQVNWEQQDQLLAIGNADLGWHISPSFKDRVAPGPGLGLTLQSLTVNDTGEYFCIYHTYPDGTYTGRIFLEVLESSVAEHGARFQIP

SEQ ID NO: 25 - protein, 120 aa, synthetic construct
MMTGTIETTGNISAEKGGSIILQCHLSSTTAQVTQVNWEQQDQLLAIINADLGWHISPSFKDRVAPGPGLGLTLQSLTVNDTGEYFCIYHTYPDGTYTGRIFLEVLESSVAEHGARFQIP

SEQ ID NO: 26 - protein, 61 aa, synthetic construct
VTQVNWEQQDQLLAIWNADLGWHISPSFKDRVAPGPGLGLTLQSLTVNDTGEYFCIYHTYP

SEQ ID NO: 27 - protein, 240 aa, synthetic construct
DIQDIQLTQSPSSLSASVGDRVTITCSASSSVRFIHWYQQKPGKAPKRLIYDTSKLASGVPSRFSGSGSGTDFTLTISSLQPEDFATYYCQQWSSSPFTFGQGTKVEIKGSTSGSGKPGSGEGSTKGSEVQLVESGGGLVQPGGSLRLSCAASGFNIKDYYIHWVRQAPGKGLEWVAWIDPENGDTEFVPKFQGRATISADTSKNTAYLQMNSLRAEDTAVYYCKTGGFWGQGTLVTVSS

SEQ ID NO: 28 - protein, 244 aa, synthetic construct
DIVMTQSPSSLSASVGDRVTVTCRASQGILTYLAWYQQKPGKAPNLLIYAASTLQSGVPSRFSGSGSGTDFTLTISSLQPEDFATYYCLQDYNFPRTFGQGTKLEIKRGSTSGSGKPGSGEGSTKGEVQLQQSGPEVKKPGASVKVSCKASGYTFTDYYMNWVRQMHGKGLEWMGVINPYNGGTDYNQKFKGRVTITADKSTSTAYMELSSLRSEDTAVYYCARSVYDYPFDYWGQGTLVTVSS

SEQ ID NO: 29 - protein, 247 aa, synthetic construct
DIQMTQSPSSLSASVGDRVTITCSTSSSVSYMHWYQQKPGKAPRLLIYSTSNLASGVPSRFSGSGSGTDFTFTISSLQPEDIATYYCHQWSSYPTFGQGTKVEIKGSTSGSGKPGSGEGSTKGQVQLQESGPGLVRPSQTLSLTCTVSGFTISSGYSWHWVRQPPGRGLEWIGYIQYSGITNYNPSLKSRVTMLVDTSKNQFSLRLSSVTAADTAVYYCAREDYDYHWYFDVWGQGSTVTVSSGAAA

SEQ ID NO: 30 - protein, 254 aa, synthetic construct
ETTLTQSPGTLSLSPGERATLSCRASQSVSSNLAWYQQKPGQAPRLLIYGASTRATGIPARFSGSGSGTEFTLTISRLEPEDFAVYYCQQRSNWPPALTFGGGTKLELKRGSTSGSGKPGSGEGSTKGQVQLQQSGAEVKKPGESLRISCKGSGYSFTSYWIGWVRQMPGKGLEWMGIIYPGDSDTRYSPSFEGQVTISADRSISTAYLQWSSLKASDTAMYYCARIRFDKEQLFYYYYGMDVWGQGTTVTVSS

SEQ ID NO: 31 - protein, 22 aa, synthetic construct
GSGATNFSLLKQAGDVEENPGP

SEQ ID NO: 32 - protein, 45 aa, synthetic construct
TTTPAPRPPTPAPTIASQPLSLRPEACRPAAGGAVHTRGLDFACD

SEQ ID NO: 33 - protein, 36 aa, synthetic construct
APPRASALPAPPTGSALPDPQTASALPDPPAASALP

SEQ ID NO: 34 - protein, 229 aa, synthetic construct
ESKYGPPCPPCPAPEFLGGPSVFLFPPKPKDTLMISRTPEVTCVVVDVSQEDPEVQFNWYVDGVEVHNAKTKPREEQFNSTYRVVSVLTVLHQDWLNGKEYKCKVSNKGLPSSIEKTISKAKGQPREPQVYTLPPSQEEMTKNQVSLTCLVKGFYPSDIAVEWESNGQPENNYKTTPPVLDSDGSFFLYSRLTVDKSRWQEGNVFSCSVMHEALHNHYTQKSLSLSLGK

SEQ ID NO: 35 - protein, 21 aa, synthetic construct
IYIWAPLAGTCGVLLLSLVIT

SEQ ID NO: 36 - protein, 27 aa, synthetic construct
FWVLVVVGGVLACYSLLVTVAFIIFWV

SEQ ID NO: 37 - protein, 41 aa, synthetic construct
RSKRSRGGHSDYMNMTPRRPGPTRKHYQPYAPPRDFAAYRS

SEQ ID NO: 38 - protein, 45 aa, synthetic construct
LYCKRGRKKLLYIFKQPFMRPVQTTQEEDGCSCRFPEEEEGGCEL

SEQ ID NO: 39 - protein, 120 aa, synthetic construct
WRRKRKEKQSETSPKEFLTIYEDVKDLKTRRNHEQEQTFPGGGSTIYSMIQSQSSAPTSQEPAYTLYSLIQPSRKSGSRKRNHSPSFNSTIYEVIGKSQPKAQNPARLSRKELENFDVYS

SEQ ID NO: 40 - protein, 84 aa, synthetic construct
RSKRSRGGHSDYMNMTPRRPGPTRKHYQPYAPPRDFAAYRSVKRGRKKLLYIFKQPFMRPVQTTQEEDGCSCRFPEEEEGGCEL

SEQ ID NO: 41 - protein, 112 aa, synthetic construct
RVKFSRSADAPAYKQGQNQLYNELNLGRREEYDVLDKRRGRDPEMGGKPRRKNPQEGLYNELQKDKMAEAYSEIGMKGERRRGKGHDGLYQGLSTATKDTYDALHMQALPPR

SEQ ID NO: 42 - protein, 112 aa, synthetic construct
RVKFSRSADAPAYQQGQSQLYNELNLGRREEYDVLDKRRGRDPEMGGKPRRKNPQEGLYNELQKDKMAEAYSEIGMKGERRRGKGHDGLYQGLSTATKDTYDALHMQALPPR

SEQ ID NO: 43 - protein, 112 aa, synthetic construct
RVKFSRSADAPAYQQGQNQLYNELNLGRREEYDVLDKRRGRDPEMGGKPRRKNPQEGLYNELQKDKMAEAYSEIGMKGERRRGKGHDGLYQGLSTATKDTYDALHMQALPPR

SEQ ID NO: 44 - protein, 21 aa, synthetic construct
FWLPIGCAAFVVVCILGCILI

SEQ ID NO: 45 - protein, 42 aa, synthetic construct
ALYLLRRDQRLPPDAHKPPGGGSFRTPIQEEQADAHSTLAKI

SEQ ID NO: 46 - protein, 38 aa, synthetic construct
CWLTKKKYSSSVHDPNGEYMFMRAVNTAKKSRLTDVTL

SEQ ID NO: 47 - protein, 120 aa, synthetic construct
MMTGTIETTGNISAEKGGSIFLQCHLSSTTAQVSQVNWKQQDQLLAIWNADLGWHISPSFKDRVAPGPGPGLTLQSLTVYDTGEYFCIYHTYPDGTYTGRTFLEVLESSAAEHGARFQIP

SEQ ID NO: 48 - protein, 120 aa, synthetic construct
MMTGTIETTGNISAEKGGSIILQCHLSSTTAQVTQVNWEQQDQLLAIWNADLGWHIPPSFKDRVAPGPGLGLTLQSLTVNDTGEYSCIYHTYPDGTYTGRIFLEVLESSVAEHGARFQIP

SEQ ID NO: 49 - protein, 120 aa, synthetic construct
MMTGTIETSGNISAEKGGSIILQCHLSSTTAQVTQVNWVQQDQLLAIWNADLGWHISPSFRDRVAPGPGLGLTLQSLTVNDTGEYFCIYHTYPDGTYTGRTFLEVLESSVAEHGARFQIP

SEQ ID NO: 50 - protein, 120 aa, synthetic construct
MMTGTIETTGNISAEKGGSTILQCHLSSTTAQVTQVNWKQQDQLLAIWNADLGWHISPSFKDRVAPGPGLGLTLQSLTVNDTGEYFCIYHTYPDGTYTGRIFLEVLESSVAEHGARFQIP

SEQ ID NO: 51 - protein, 120 aa, synthetic construct
MMTGTIETTGNISAEKGGSIILQCHLSSTTAQVTQVNWEQQDQLLAIWNADLGWHISPSFKDRVAPGPGLDLTLQSLTVNDTGEYFCVYHTYPDGTYTGRIFLEVLESSVAEHGARFQIP

SEQ ID NO: 52 - protein, 61 aa, synthetic construct
VTQVNWEQQDQLLAIWNADLGWHIPPSFKDRVAPGPGLGLTLQSLTVNDTGEYSCIYHTYP

SEQ ID NO: 53 - protein, 61 aa, synthetic construct
VTQVNWEQQDQLLAIWNADLGWHISPSFKDRVAPGPGLDLTLQSLTVNDTGEYFCVYHTYP